European Patent Specification EP 4 077 344 B1, published July 23, 2025. Title: METHODS OF SEQUENCING BY SYNTHESIS USING A CONSECUTIVE LABELING SCHEME. Applicant: ROCHE SEQUENCING SOLUTIONS, INC. F. HOFFMANN-LA ROCHE AG ROCHE DIAGNOSTICS GMBH. The sequence listing filed with the application follows.

SEQUENCE LISTING (58 sequences)

SEQ ID NO: 1 - DNA, 5 bp, Artificial Sequence
  Synthetic
cttcc

SEQ ID NO: 2 - DNA, 5 bp, Artificial Sequence
  Synthetic
gctcc

SEQ ID NO: 3 - DNA, 6 bp, Artificial Sequence
  Synthetic
gttggt

SEQ ID NO: 4 - DNA, 6 bp, Artificial Sequence
  Synthetic
ctgtca

SEQ ID NO: 5 - DNA, 6 bp, Artificial Sequence
  Synthetic
tgctcc

SEQ ID NO: 6 - DNA, 6 bp, Artificial Sequence
  Synthetic
tcttcc

SEQ ID NO: 7 - DNA, 8 bp, Artificial Sequence
  Synthetic
gttggtgt

SEQ ID NO: 8 - DNA, 7 bp, Artificial Sequence
  Synthetic
gttggtg

SEQ ID NO: 9 - DNA, 8 bp, Artificial Sequence
  Synthetic
tgctcctg

SEQ ID NO: 10 - DNA, 8 bp, Artificial Sequence
  Synthetic
gtgcgtct

SEQ ID NO: 11 - DNA, 8 bp, Artificial Sequence
  Synthetic
gttggtgt

SEQ ID NO: 12 - DNA, 9 bp, Artificial Sequence
  Synthetic
tgctcctgt

SEQ ID NO: 13 - DNA, 9 bp, Artificial Sequence
  Synthetic
gttggtgtg

SEQ ID NO: 14 - DNA, 9 bp, Artificial Sequence
  Synthetic
ttctcttcc

SEQ ID NO: 15 - DNA, 12 bp, Artificial Sequence
  Synthetic
gttggtgtgttg

SEQ ID NO: 16 - DNA, 15 bp, Artificial Sequence
  Synthetic
gttggtgtgttggtg

SEQ ID NO: 17 - DNA, 9 bp, Artificial Sequence
  Synthetic
aaaaaaaaa

SEQ ID NO: 18 - DNA, 6 bp, Artificial Sequence
  Synthetic
aaaaaa

SEQ ID NO: 19 - DNA, 6 bp, Artificial Sequence
  Synthetic
tatcgc

SEQ ID NO: 20 - DNA, 6 bp, Artificial Sequence
  Synthetic
tctgac

SEQ ID NO: 21 - DNA, 6 bp, Artificial Sequence
  Synthetic
agagag

SEQ ID NO: 22 - DNA, 6 bp, Artificial Sequence
  Synthetic
cacaca

SEQ ID NO: 23 - DNA, 20 bp, Artificial Sequence
  Synthetic
cagtggacgacgatagacat

SEQ ID NO: 24 - DNA, 20 bp, Artificial Sequence
  Synthetic
agaggatcgaggagtacagg

SEQ ID NO: 25 - DNA, 20 bp, Artificial Sequence
  Synthetic
agaaatggacgagatgctaa

SEQ ID NO: 26 - DNA, 20 bp, Artificial Sequence
  Synthetic
actgaacttgtgagaaacgc

SEQ ID NO: 27 - DNA, 20 bp, Artificial Sequence
  Synthetic
atggagagtcaggcaagttt

SEQ ID NO: 28 - DNA, 20 bp, Artificial Sequence
  Synthetic
tgaagatgcgagtgatgaac

SEQ ID NO: 29 - DNA, 5 bp, Artificial Sequence
  Synthetic
ggaag

SEQ ID NO: 30 - DNA, 5 bp, Artificial Sequence
  Synthetic
ggagc

SEQ ID NO: 31 - DNA, 6 bp, Artificial Sequence
  Synthetic
accaac

SEQ ID NO: 32 - DNA, 6 bp, Artificial Sequence
  Synthetic
tgacag

SEQ ID NO: 33 - DNA, 6 bp, Artificial Sequence
  Synthetic
ggagca

SEQ ID NO: 34 - DNA, 6 bp, Artificial Sequence
  Synthetic
ggaaga

SEQ ID NO: 35 - DNA, 8 bp, Artificial Sequence
  Synthetic
acaccaac

SEQ ID NO: 36 - DNA, 7 bp, Artificial Sequence
  Synthetic
caccaac

SEQ ID NO: 37 - DNA, 8 bp, Artificial Sequence
  Synthetic
caggagca

SEQ ID NO: 38 - DNA, 8 bp, Artificial Sequence
  Synthetic
agacgcac

SEQ ID NO: 39 - DNA, 8 bp, Artificial Sequence
  Synthetic
acaccaac

SEQ ID NO: 40 - DNA, 9 bp, Artificial Sequence
  Synthetic
acaggagca

SEQ ID NO: 41 - DNA, 9 bp, Artificial Sequence
  Synthetic
cacaccaac

SEQ ID NO: 42 - DNA, 9 bp, Artificial Sequence
  Synthetic
ggaagagaa

SEQ ID NO: 43 - DNA, 12 bp, Artificial Sequence
  Synthetic
caacacaccaac

SEQ ID NO: 44 - DNA, 15 bp, Artificial Sequence
  Synthetic
caccaacacaccaac

SEQ ID NO: 45 - DNA, 9 bp, Artificial Sequence
  Synthetic
ttttttttt

SEQ ID NO: 46 - DNA, 6 bp, Artificial Sequence
  Synthetic
tttttt

SEQ ID NO: 47 - DNA, 6 bp, Artificial Sequence
  Synthetic
gcgata

SEQ ID NO: 48 - DNA, 6 bp, Artificial Sequence
  Synthetic
gtcaga

SEQ ID NO: 49 - DNA, 6 bp, Artificial Sequence
  Synthetic
ctctct

SEQ ID NO: 50 - DNA, 6 bp, Artificial Sequence
  Synthetic
tgtgtg

SEQ ID NO: 51 - DNA, 20 bp, Artificial Sequence
  Synthetic
atgtctatcgtcgtccactg

SEQ ID NO: 52 - DNA, 20 bp, Artificial Sequence
  Synthetic
cctgtactcctcgatcctct

SEQ ID NO: 53 - DNA, 20 bp, Artificial Sequence
  Synthetic
ttagcatctcgtccatttct

SEQ ID NO: 54 - DNA, 20 bp, Artificial Sequence
  Synthetic
gcgtttctcacaagttcagt

SEQ ID NO: 55 - DNA, 20 bp, Artificial Sequence
  Synthetic
aaacttgcctgactctccat

SEQ ID NO: 56 - DNA, 20 bp, Artificial Sequence
  Synthetic
gttcatcactcgcatcttca

SEQ ID NO: 57 - DNA, 6 bp, Artificial Sequence
  Synthetic
tgagtg

SEQ ID NO: 58 - DNA, 6 bp, Artificial Sequence
  Synthetic
cactca